European Patent Application EP 4 191 638 A1, published June 7, 2023. Title: SURFACE LINKER OF SEMICONDUCTOR CHIP, PREPARATION METHOD THEREFOR AND APPLICATION THEREOF. Applicant: Nanjing GenScript Biotech Co., Ltd. The sequence listing filed with the application follows.

SEQUENCE LISTING (3 sequences)

SEQ ID NO: 1 - DNA, 38 bp, Artificial Sequence
  DNA-H1
  NH2 (38)..(38)
acactctttccctacacgacgctcttccgatctttttt

SEQ ID NO: 2 - DNA, 14 bp, Artificial Sequence
  DNA-H2-cy5
  Cy5 (14)..(14)
tagggaaagagtgt

SEQ ID NO: 3 - DNA, 14 bp, Artificial Sequence
  DNA-H2-cy3
  Cy3 (14)..(14)
agatcggaagagcg